European Patent Application EP 4 625 419 A1, published October 1, 2025. Title: CODON OPTIMIZATION. Applicant: NANJING GENSCRIPT BIOTECH CO., LTD. The sequence listing filed with the application follows.

SEQUENCE LISTING (3 sequences)

SEQ ID NO: 1 - protein, 190 aa, synthetic construct
MSRKAPCKYEVRGKCNRGSECKFNHNYWSWPDRYLLLRSNYLLNQLLRNTDRSDGLSLISGAGRDDRTQDFVLGSTNVVQNYIDNNENITKASACYSLYNIIKQLQETDVRQARDNKVDDSKHVALHNLVLSYMEMSKTPASLINNLKKPPKEKLKKLAKLIIELSAGVENDSTAAMQDSANSDHHHHHH

SEQ ID NO: 2 - DNA, 573 bp, synthetic construct
  source 1..573: mol_type = other DNA
atgtcaaggaaggctccctgtaaatatgaagtgcgcggcaagtgcaacagaggtagcgagtgcaagtttaatcataattactggtcttggccagatcgttatctgttgctacgcagcaactacttgttgaatcagttgctgcgtaataccgaccgtagcgacggcctgtcgctgatcagcggtgcaggtcgtgacgaccgcacccaggacttcgtgctgggttcgactaacgtggtccagaattacattgataacaacgaaaatatcaccaaagcgtctgcgtgttatagcttatataacattattaaacagctgcaagagaccgatgttcgtcaagcgcgtgacaacaaagttgatgactccaagcatgttgccctgcataacctggttctgtcctacatggaaatgagcaagaccccggcatccctgattaacaacctgaagaaaccgccgaaagaaaaactcaagaagctggcgaaactgatcatcgagctgagcgcgggcgtggagaacgattctacggctgccatgcaagacagcgctaatagcgatcaccaccaccaccaccattaa

SEQ ID NO: 3 - DNA, 573 bp, synthetic construct
  source 1..573: mol_type = other DNA
atgagccgtaaagcaccgtgtaaatatgaagttcgtggtaaatgtaatcgtggtagcgaatgtaaatttaaccataattattggagctggcctgatcgttatctgctgctgcgtagcaattatctgctgaatcagctgctgcgtaataccgatcgttcagatggtctgagcctgattagcggtgcaggtcgtgatgatcgtacccaggattttgttctgggtagcaccaatgttgttcagaactatatcgataacaacgaaaacattaccaaagcaagcgcatgttatagcctgtataacattattaaacagctgcaagaaaccgatgttcgtcaggcacgtgataataaagttgatgatagcaaacatgttgccctgcataatctggttctgagctatatggaaatgagcaaaacaccggcaagcctgattaataacctgaaaaaaccgcctaaagaaaaactgaaaaaactggcaaaactgattattgaactgagcgcaggtgttgaaaatgatagcaccgcagcaatgcaggatagcgcaaatagcgatcatcatcatcatcatcattaa